European Patent Application EP 4 471 062 A1, published December 4, 2024. Title: ANTI-CD73 ANTIBODY AND USE THEREOF. Applicant: CSPC Megalith Biopharmaceutical Co., Ltd. The sequence listing filed with the application follows.

SEQUENCE LISTING (42 sequences)

SEQ ID NO: 1 - protein, 5 aa, synthetic construct
SYDIN

SEQ ID NO: 2 - protein, 17 aa, synthetic construct
WIYPRDGFTKYNEKFKG

SEQ ID NO: 3 - protein, 12 aa, synthetic construct
KEGYRGDWYFDV

SEQ ID NO: 4 - protein, 121 aa, synthetic construct
QVQLQQSGPELVKPGASVKLSCKASGYTFTSYDINWVKQRPGQGLEWIGWIYPRDGFTKYNEKFKGKATLTVDTSSSTAYMELHSLTSEDSAVYFCARKEGYRGDWYFDVWGTGTTVTVSS

SEQ ID NO: 5 - protein, 11 aa, synthetic construct
RASGNVHNYLA

SEQ ID NO: 6 - protein, 7 aa, synthetic construct
NAKTLAD

SEQ ID NO: 7 - protein, 9 aa, synthetic construct
QHFWSTPWT

SEQ ID NO: 8 - protein, 107 aa, synthetic construct
DIQMTQSPASLSASVGETVTITCRASGNVHNYLAWYQQKQGKSPQLLVYNAKTLADGVPSRFSGSGSGTQYSLKINSLQPEDFGSYYCQHFWSTPWTFGGGTELEIK

SEQ ID NO: 9 - protein, 5 aa, synthetic construct
SYWMH

SEQ ID NO: 10 - protein, 17 aa, synthetic construct
NINPSNGGTKYNEKFKS

SEQ ID NO: 11 - protein, 8 aa, synthetic construct
RDYGSPSY

SEQ ID NO: 12 - protein, 117 aa, synthetic construct
QVQLQQPGTELVKPGASVKLSCKASGYTFTSYWMHWVKQRPGHGLEWIGNINPSNGGTKYNEKFKSKATLTVDKSSSTAYLQLSSLTSEDSAVYYCARRDYGSPSYWGQGTLVTVSA

SEQ ID NO: 13 - protein, 11 aa, synthetic construct
KASQDINSYLT

SEQ ID NO: 14 - protein, 7 aa, synthetic construct
RTNILLD

SEQ ID NO: 15 - protein, 9 aa, synthetic construct
LQYHEFPVT

SEQ ID NO: 16 - protein, 107 aa, synthetic construct
DIKMTQSPSSIYASLGERVTITCKASQDINSYLTWFQQKVGKSPKTLIYRTNILLDGVPSRFSGSGSGQDYSLTISSLDYEDMGIYHCLQYHEFPVTFGAGTKLELK

SEQ ID NO: 17 - protein, 17 aa, synthetic construct
WIYPRDGFTGYAQKFQG

SEQ ID NO: 18 - protein, 121 aa, synthetic construct
QVQLVQSGAEVKKPGASVKVSCKASGYTFTSYDINWVRQATGQGLEWMGWIYPRDGFTGYAQKFQGRVTITRNTSISTAYMELSSLRSEDTAVYYCARKEGYRGDWYFDVWGQGTTVTVSS

SEQ ID NO: 19 - protein, 121 aa, synthetic construct
QVQLVQSGAEVKKPGASVKLSCKASGYTFTSYDINWVRQATGQGLEWIGWIYPRDGFTKYNEKFKGRATLTVDTSISTAYMELSSLRSEDTAVYYCARKEGYRGDWYFDVWGQGTTVTVSS

SEQ ID NO: 20 - protein, 121 aa, synthetic construct
QVQLVQSGAEVKKPGASVKVSCKASGYTFTSYDINWVRQATGQGLEWIGWIYPRDGFTKYNEKFKGRVTLTVNTSISTAYMELSSLRSEDTAVYYCARKEGYRGDWYFDVWGQGTTVTVSS

SEQ ID NO: 21 - protein, 17 aa, synthetic construct
WIYPRDGFTKYNEKFQG

SEQ ID NO: 22 - protein, 121 aa, synthetic construct
QVQLVQSGAEVKKPGASVKVSCKASGYTFTSYDINWVRQATGQGLEWIGWIYPRDGFTKYNEKFQGRVTITVNTSISTAYMELSSLRSEDTAVYYCARKEGYRGDWYFDVWGQGTTVTVSS

SEQ ID NO: 23 - protein, 17 aa, synthetic construct
WIYPRDGFTKYAQKFQG

SEQ ID NO: 24 - protein, 121 aa, synthetic construct
QVQLVQSGAEVKKPGASVKVSCKASGYTFTSYDINWVRQATGQGLEWMGWIYPRDGFTKYAQKFQGRVTITVNTSISTAYMELSSLRSEDTAVYYCARKEGYRGDWYFDVWGQGTTVTVSS

SEQ ID NO: 25 - protein, 117 aa, synthetic construct
QVQLVQSGAEVKKPGASVKLSCKASGYTFTSYWMHWVRQAPGQRLEWIGNINPSNGGTKYNEKFKSRATLTVDKSASTAYLELSSLRSEDTAVYYCARRDYGSPSYWGQGTTVTVSS

SEQ ID NO: 26 - protein, 117 aa, synthetic construct
QVQLVQSGAEVKKPGASVKVSCKASGYTFTSYWMHWVRQAPGQRLEWIGNINPSNGGTKYNEKFKSRVTITVDKSASTAYLELSSLRSEDTAVYYCARRDYGSPSYWGQGTTVTVSS

SEQ ID NO: 27 - protein, 17 aa, synthetic construct
NINPSNGGTKYNEKFQG

SEQ ID NO: 28 - protein, 117 aa, synthetic construct
QVQLVQSGAEVKKPGASVKVSCKASGYTFTSYWMHWVRQAPGQRLEWIGNINPSNGGTKYNEKFQGRVTITVDTSASTAYLELSSLRSEDTAVYYCARRDYGSPSYWGQGTTVTVSS

SEQ ID NO: 29 - protein, 117 aa, synthetic construct
QVQLVQSGAEVKKPGASVKVSCKASGYTFTSYWMHWVRQAPGQRLEWMGNINPSNGGTKYNEKFQGRVTITVDTSASTAYMELSSLRSEDTAVYYCARRDYGSPSYWGQGTTVTVSS

SEQ ID NO: 30 - protein, 17 aa, synthetic construct
NINPSNGGTKYSQKFQG

SEQ ID NO: 31 - protein, 117 aa, synthetic construct
QVQLVQSGAEVKKPGASVKVSCKASGYTFTSYWMHWVRQAPGQRLEWMGNINPSNGGTKYSQKFQGRVTITVDTSASTAYMELSSLRSEDTAVYYCARRDYGSPSYWGQGTTVTVSS

SEQ ID NO: 32 - protein, 7 aa, synthetic construct
NAKTLAS

SEQ ID NO: 33 - protein, 107 aa, synthetic construct
DIQMTQSPSSLSASVGDRVTITCRASGNVHNYLAWYQQKPGKAPKLLLYNAKTLASGVPSRFSGSGSGTDYTLTISSLQPEDFATYYCQHFWSTPWTFGGGTELEIK

SEQ ID NO: 34 - protein, 107 aa, synthetic construct
DIQMTQSPSSLSASVGDRVTITCRASGNVHNYLAWYQQKPGKAPKLLVYNAKTLADGVPSRFSGSGSGTDYTLTISSLQPEDFATYYCQHFWSTPWTFGGGTELEIK

SEQ ID NO: 35 - protein, 11 aa, synthetic construct
RASQDINSYLT

SEQ ID NO: 36 - protein, 107 aa, synthetic construct
DIQMTQSPSSLSASVGDRVTITCRASQDINSYLTWFQQKPGKAPKSLIYRTNILLDGVPSRFSGSGSGTDFTLTISSLQPEDFATYYCLQYHEFPVTFGGGTKLEIK

SEQ ID NO: 37 - protein, 107 aa, synthetic construct
DIKMTQSPSSLSASVGDRVTITCKASQDINSYLTWFQQKVGKAPKTLIYRTNILLDGVPSRFSGSGSGTDYTLTISSLQPEDFATYHCLQYHEFPVTFGGGTKLEIK

SEQ ID NO: 38 - protein, 107 aa, synthetic construct
DIQMTQSPSSLSASVGDRVTITCKASQDINSYLTWFQQKPGKAPKSLIYRTNILLDGVPSRFSGSGSGTDYTLTISSLQPEDFATYYCLQYHEFPVTFGGGTKLEIK

SEQ ID NO: 39 - protein, 330 aa, synthetic construct
ASTKGPSVFPLAPSSKSTSGGTAALGCLVKDYFPEPVTVSWNSGALTSGVHTFPAVLQSSGLYSLSSVVTVPSSSLGTQTYICNVNHKPSNTKVDKKVEPKSCDKTHTCPPCPAPEAAGGPSVFLFPPKPKDTLMISRTPEVTCVVVDVSHEDPEVKFNWYVDGVEVHNAKTKPREEQYNSTYRVVSVLTVLHQDWLNGKEYKCKVSNKALAASIEKTISKAKGQPREPQVYTLPPSRDELTKNQVSLTCLVKGFYPSDIAVEWESNGQPENNYKTTPPVLDSDGSFFLYSKLTVDKSRWQQGNVFSCSVMHEALHNHYTQKSLSLSPGK

SEQ ID NO: 40 - protein, 107 aa, synthetic construct [sequence omitted]

SEQ ID NO: 41 - protein, 213 aa, Homo sapiens
QELGKTIVYLDGSSQSCRFRECNMGNLICDAMINNNLRHTDEMFWNHVSMCILNGGGIRSPIDERNNGTITWENLAAVLPFGGTFDLVQLKGSTLKKAFEHSVHRYGQSTGEFLQVGGIHVVYDLSRKPGDRVVKLDVLCTKCRVPSYDPLKMDEVYKVILPNFLANGGDGFQMIKDELLRHDSGDQDINVVSTYISKMKVIYPAVEGRIKFS

SEQ ID NO: 42 - protein, 317 aa, Homo sapiens
MCPRAARAPATLLLALGAVLWPAAGAWELTILHTNDVHSRLEQTSEDSSKCVNASRCMGGVARLFTKVQQIRRAEPNVLLLDAGDQYQGTIWFTVYKGAEVAHFMNALRYDAMALGNHEFDNGVEGLIEPLLKEAKFPILSANIKAKGPLASQISGLYLPYKVLPVGDEVVGIVGYTSKETPFLSNPGTNLVFEDEITALQPEVDKLKTLNVNKIIALGHSGFEMDKLIAQKVRGVDVVVGGHSNTFLYTGNPPSKEVPAGKYPFIVTSDDGRKVPVVQAYAFGKYLGYLKIEFDERGNVISSHGNPILLNSSIPED